European Patent Application EP 4 556 486 A1, published May 21, 2025. Title: TRISPECIFIC ANTIBODY AND USE THEREOF. Applicant: CYTOCARES (SHANGHAI) INC. Application EP EP23838948.0, filed July 11, 2023. The sequence listing filed with the application follows.

SEQUENCE LISTING (69 sequences)

SEQ ID NO: 1 - protein, 15 aa, synthetic construct
GGGGSGGGGSGGGGS

SEQ ID NO: 2 - protein, 5 aa, synthetic construct
GGGGS

SEQ ID NO: 3 - protein, 14 aa, synthetic construct
GGSGGSGGSGGSGG

SEQ ID NO: 4 - protein, 81 aa, synthetic construct
ASKSKKEIFRWPESPKAQASSVPTAQPQAEGSLAKATTAPATTRNTGRGGEEKKKEKEKEEQEERETKTPESPSHTQPLGV

SEQ ID NO: 5 - protein, 38 aa, synthetic construct
RNTGRGGEEKKKEKEKEEQEERETKTPECPSHTQPLGV

SEQ ID NO: 6 - protein, 38 aa, synthetic construct
RNTGRGGEEKKKEKEKEEQEERETKTPESPSHTQPLGV

SEQ ID NO: 7 - protein, 5 aa, synthetic construct
EAAAK

SEQ ID NO: 8 - protein, 81 aa, synthetic construct
ASKSKKEIFRWPESPKAQASSVPTAQPQAEGSLAKATTAPATTRNTGRGGEEKKKEKEKEEQEERETKTPEGPSHTQPLGV

SEQ ID NO: 9 - protein, 38 aa, synthetic construct
RNTGRGGEEKKKEKEKEEQEERETKTPEGPSHTQPLGV

SEQ ID NO: 10 - protein, 81 aa, synthetic construct
ASKSKKEIFRWPESPKAQASSVPTAQPQAEGSLAKATTAPATTRNTGRGGEEKKKEKEKEEQEERETKTPECPSHTQPLGV

SEQ ID NO: 11 - protein, 5 aa, synthetic construct
SYWMN

SEQ ID NO: 12 - protein, 17 aa, synthetic construct
QIWPGDGDTNYNGKFKG

SEQ ID NO: 13 - protein, 15 aa, synthetic construct
RETTTVGRYYYAMDY

SEQ ID NO: 14 - protein, 15 aa, synthetic construct
KASQSVDYDGDSYLN

SEQ ID NO: 15 - protein, 7 aa, synthetic construct
DASNLVS

SEQ ID NO: 16 - protein, 9 aa, synthetic construct
QQSTEDPWT

SEQ ID NO: 17 - protein, 124 aa, synthetic construct
QVQLQQSGAELVRPGSSVKISCKASGYAFSSYWMNWVKQRPGQGLEWIGQIWPGDGDTNYNGKFKGKATLTADESSSTAYMQLSSLASEDSAVYFCARRETTTVGRYYYAMDYWGQGTTVTVSS

SEQ ID NO: 18 - DNA, 372 bp, synthetic construct
  source 1..372: mol_type = other DNA
caggtgcagctccagcagtctggagcagagctggtgcggcccggcagcagcgtcaagatttcctgtaaagcatctgggtatgccttttctagttactggatgaattgggtgaagcagagacccggccagggactggagtggattggacagatttggcctggggatggtgacaccaactacaatggcaagttcaaaggcaaggctaccctgacagcagacgaatcaagctccacagcttacatgcagctgtctagtctggcatcagaggatagcgccgtgtatttttgcgctcggagggaaaccacaactgtcggccgctactattacgctatggactactggggccagggaaccacagtgacagtctcaagc

SEQ ID NO: 19 - protein, 111 aa, synthetic construct
DIQLTQSPASLAVSLGQRATISCKASQSVDYDGDSYLNWYQQIPGQPPKLLIYDASNLVSGIPPRFSGSGSGTDFTLNIHPVEKVDAATYHCQQSTEDPWTFGGGTKLEIK

SEQ ID NO: 20 - DNA, 333 bp, synthetic construct
  source 1..333: mol_type = other DNA
gacatccagctgacacagtctccagctagtctggcagtgagcctgggacagagagctactatttcctgcaaggcaagccagtccgtggactacgatggagactcctatctgaactggtatcagcagatccccggccagccccctaaactgctgatttatgatgcttcaaatctggtgagcggcatcccaccccgcttctctggaagtgggtcaggcaccgattttacactgaacattcaccccgtggagaaggtggacgccgctacctaccattgccagcagtccactgaggacccctggaccttcggcggcggcaccaagctggaaatcaaa

SEQ ID NO: 21 - protein, 250 aa, synthetic construct
DIQLTQSPASLAVSLGQRATISCKASQSVDYDGDSYLNWYQQIPGQPPKLLIYDASNLVSGIPPRFSGSGSGTDFTLNIHPVEKVDAATYHCQQSTEDPWTFGGGTKLEIKGGGGSGGGGSGGGGSQVQLQQSGAELVRPGSSVKISCKASGYAFSSYWMNWVKQRPGQGLEWIGQIWPGDGDTNYNGKFKGKATLTADESSSTAYMQLSSLASEDSAVYFCARRETTTVGRYYYAMDYWGQGTTVTVSS

SEQ ID NO: 22 - protein, 5 aa, synthetic construct
RYTMH

SEQ ID NO: 23 - protein, 17 aa, synthetic construct
YINPSRGYTNYNQKFKD

SEQ ID NO: 24 - protein, 10 aa, synthetic construct
YYDDHYCLDY

SEQ ID NO: 25 - protein, 10 aa, synthetic construct
RASSSVSYMN

SEQ ID NO: 26 - protein, 7 aa, synthetic construct
DTSKVAS

SEQ ID NO: 27 - protein, 9 aa, synthetic construct
QQWSSNPLT

SEQ ID NO: 28 - protein, 121 aa, synthetic construct
DIKLQQSGAELARPGASVKMSCKTSGYTFTRYTMHWVKQRPGQGLEWIGYINPSRGYTNYNQKFKDKATLTTDKSSSTAYMQLSSLTSEDSAVYYCARYYDDHYCLDYWGQGTTLTVSSVE

SEQ ID NO: 29 - DNA, 363 bp, synthetic construct
  source 1..363: mol_type = other DNA
gacatcaagctccagcagtctggtgccgagctggctcgaccaggagccagtgtgaagatgtcatgtaaaaccagtggctatactttcaccagatacacaatgcactgggtgaaacagcgcccagggcagggtctggaatggatcgggtacattaaccccagccggggctacaccaactacaaccagaagttcaaggataaagccactctgactaccgacaagtcctctagtaccgcttatatgcagctgtcaagcctgacatccgaggacagcgccgtgtactactgcgccaggtattacgacgatcattattgtctggattactggggccagggaacaactctgaccgtgagcagcgtcgaa

SEQ ID NO: 30 - protein, 108 aa, synthetic construct
VDDIQLTQSPAIMSASPGEKVTMTCRASSSVSYMNWYQQKSGTSPKRWIYDTSKVASGVPYRFSGSGSGTSYSLTISSMEAEDAATYYCQQWSSNPLTFGAGTKLELK

SEQ ID NO: 31 - DNA, 324 bp, synthetic construct
  source 1..324: mol_type = other DNA
gtggacgacatccagctgacccagtctcctgccattatgagcgccagccccggcgagaaggtgacaatgacttgccgagctagttcaagcgtcagctatatgaattggtatcagcagaaatctggcaccagccctaaacgatggatctatgacacctctaaagtggcaagcggagtcccataccggttctctgggagtggttcaggcactagctattccctgaccatttcctctatggaggcagaagatgcagccacctattactgtcagcagtggagttcaaatcccctgacatttggagccgggactaagctggagctgaaa

SEQ ID NO: 32 - protein, 243 aa, synthetic construct
DIKLQQSGAELARPGASVKMSCKTSGYTFTRYTMHWVKQRPGQGLEWIGYINPSRGYTNYNQKFKDKATLTTDKSSSTAYMQLSSLTSEDSAVYYCARYYDDHYCLDYWGQGTTLTVSSVEGGSGGSGGSGGSGGVDDIQLTQSPAIMSASPGEKVTMTCRASSSVSYMNWYQQKSGTSPKRWIYDTSKVASGVPYRFSGSGSGTSYSLTISSMEAEDAATYYCQQWSSNPLTFGAGTKLELK

SEQ ID NO: 33 - protein, 5 aa, synthetic construct
SYYIH

SEQ ID NO: 34 - protein, 17 aa, synthetic construct
CIYPGNVNTNYNEKFKD

SEQ ID NO: 35 - protein, 11 aa, synthetic construct
SHYGLDWNFDV

SEQ ID NO: 36 - protein, 11 aa, synthetic construct
HASQNIYVWLN

SEQ ID NO: 37 - protein, 7 aa, synthetic construct
KASNLHT

SEQ ID NO: 38 - protein, 9 aa, synthetic construct
QQGQTYPYT

SEQ ID NO: 39 - protein, 120 aa, synthetic construct
QVQLVQSGAEVKKPGASVKVSCKASGYTFTSYYIHWVRQAPGQGLEWIGCIYPGNVNTNYNEKFKDRATLTVDTSISTAYMELSRLRSDDTAVYFCTRSHYGLDWNFDVWGQGTTVTVSS

SEQ ID NO: 40 - DNA, 360 bp, synthetic construct
  source 1..360: mol_type = other DNA
caggtgcagctggtccagtcaggagcagaagtcaaaaaacccggcgcatcagtcaaagtctcttgtaaagcctccggatacacatttacatcctactatatccactgggtcagacaggcacctggccagggactggagtggatcggctgcatttacccaggaaacgtgaacaccaactacaacgaaaagttcaaggaccgcgctactctgaccgtcgatacatcaattagcactgcatacatggagctgtctcggctgaggagtgacgatacagctgtgtacttctgtactcgatctcattatggcctggactggaactttgatgtgtgggggcagggcaccacagtgaccgtcagctcc

SEQ ID NO: 41 - protein, 108 aa, synthetic construct
DIQMTQSPSSLSASVGDRVTITCHASQNIYVWLNWYQQKPGKAPKLLIYKASNLHTGVPSRFSGSGSGTDFTLTISSLQPEDFATYYCQQGQTYPYTFGGGTKVEIKR

SEQ ID NO: 42 - DNA, 324 bp, synthetic construct
  source 1..324: mol_type = other DNA
gacatccagatgacacagagcccttcaagcctgagcgcctccgtcggtgacagagtgaccattacctgccacgcctcccagaatatctacgtgtggctgaactggtatcagcagaagccaggcaaagcacccaagctgctgatctacaaagccagcaatctgcacaccggagtcccaagcagattctccggttctggcagtggaacagactttaccctgacaatcagcagcctccagcctgaggatttcgcaacttactattgccagcagggccagacatacccatatacttttggcggagggaccaaagtggagatcaagcgg

SEQ ID NO: 43 - protein, 243 aa, synthetic construct
QVQLVQSGAEVKKPGASVKVSCKASGYTFTSYYIHWVRQAPGQGLEWIGCIYPGNVNTNYNEKFKDRATLTVDTSISTAYMELSRLRSDDTAVYFCTRSHYGLDWNFDVWGQGTTVTVSSGGGGSGGGGSGGGGSDIQMTQSPSSLSASVGDRVTITCHASQNIYVWLNWYQQKPGKAPKLLIYKASNLHTGVPSRFSGSGSGTDFTLTISSLQPEDFATYYCQQGQTYPYTFGGGTKVEIKR

SEQ ID NO: 44 - protein, 779 aa, synthetic construct
DIQLTQSPASLAVSLGQRATISCKASQSVDYDGDSYLNWYQQIPGQPPKLLIYDASNLVSGIPPRFSGSGSGTDFTLNIHPVEKVDAATYHCQQSTEDPWTFGGGTKLEIKGGGGSGGGGSGGGGSQVQLQQSGAELVRPGSSVKISCKASGYAFSSYWMNWVKQRPGQGLEWIGQIWPGDGDTNYNGKFKGKATLTADESSSTAYMQLSSLASEDSAVYFCARRETTTVGRYYYAMDYWGQGTTVTVSSGGGGSDIKLQQSGAELARPGASVKMSCKTSGYTFTRYTMHWVKQRPGQGLEWIGYINPSRGYTNYNQKFKDKATLTTDKSSSTAYMQLSSLTSEDSAVYYCARYYDDHYCLDYWGQGTTLTVSSVEGGSGGSGGSGGSGGVDDIQLTQSPAIMSASPGEKVTMTCRASSSVSYMNWYQQKSGTSPKRWIYDTSKVASGVPYRFSGSGSGTSYSLTISSMEAEDAATYYCQQWSSNPLTFGAGTKLELKRNTGRGGEEKKKEKEKEEQEERETKTPESPSHTQPLGVQVQLVQSGAEVKKPGASVKVSCKASGYTFTSYYIHWVRQAPGQGLEWIGCIYPGNVNTNYNEKFKDRATLTVDTSISTAYMELSRLRSDDTAVYFCTRSHYGLDWNFDVWGQGTTVTVSSGGGGSGGGGSGGGGSDIQMTQSPSSLSASVGDRVTITCHASQNIYVWLNWYQQKPGKAPKLLIYKASNLHTGVPSRFSGSGSGTDFTLTISSLQPEDFATYYCQQGQTYPYTFGGGTKVEIKR

SEQ ID NO: 45 - DNA, 2400 bp, synthetic construct
  source 1..2400: mol_type = other DNA
atggccacccggctgaccgtgctggccctgctggccggcctgctggcctcctccagggccgacatccagctgacacagtctccagctagtctggcagtgagcctgggacagagagctactatttcctgcaaggcaagccagtccgtggactacgatggagactcctatctgaactggtatcagcagatccccggccagccccctaaactgctgatttatgatgcttcaaatctggtgagcggcatcccaccccgcttctctggaagtgggtcaggcaccgattttacactgaacattcaccccgtggagaaggtggacgccgctacctaccattgccagcagtccactgaggacccctggaccttcggcggcggcaccaagctggaaatcaaaggtggcggagggtccggtggcggagggtctggtggcggagggagccaggtgcagctccagcagtctggagcagagctggtgcggcccggcagcagcgtcaagatttcctgtaaagcatctgggtatgccttttctagttactggatgaattgggtgaagcagagacccggccagggactggagtggattggacagatttggcctggggatggtgacaccaactacaatggcaagttcaaaggcaaggctaccctgacagcagacgaatcaagctccacagcttacatgcagctgtctagtctggcatcagaggatagcgccgtgtatttttgcgctcggagggaaaccacaactgtcggccgctactattacgctatggactactggggccagggaaccacagtgacagtctcaagcggtggcggagggtccgacatcaagctccagcagtctggtgccgagctggctcgaccaggagccagtgtgaagatgtcatgtaaaaccagtggctatactttcaccagatacacaatgcactgggtgaaacagcgcccagggcagggtctggaatggatcgggtacattaaccccagccggggctacaccaactacaaccagaagttcaaggataaagccactctgactaccgacaagtcctctagtaccgcttatatgcagctgtcaagcctgacatccgaggacagcgccgtgtactactgcgccaggtattacgacgatcattattgtctggattactggggccagggaacaactctgaccgtgagcagcgtcgaaggtggcagtggagggtcaggtggcagcggagggtccggtggcgtggacgacatccagctgacccagtctcctgccattatgagcgccagccccggcgagaaggtgacaatgacttgccgagctagttcaagcgtcagctatatgaattggtatcagcagaaatctggcaccagccctaaacgatggatctatgacacctctaaagtggcaagcggagtcccataccggttctctgggagtggttcaggcactagctattccctgaccatttcctctatggaggcagaagatgcagccacctattactgtcagcagtggagttcaaatcccctgacatttggagccgggactaagctggagctgaaaagaaataccggcagaggcggagaggagaagaagaaggagaaggagaaggaggagcaggaggagagagagaccaagacacccgagtctcctagccacacacagcctctgggagtgcaggtgcagctggtccagtcaggagcagaagtcaaaaaacccggcgcatcagtcaaagtctcttgtaaagcctccggatacacatttacatcctactatatccactgggtcagacaggcacctggccagggactggagtggatcggctgcatttacccaggaaacgtgaacaccaactacaacgaaaagttcaaggaccgcgctactctgaccgtcgatacatcaattagcactgcatacatggagctgtctcggctgaggagtgacgatacagctgtgtacttctgtactcgatctcattatggcctggactggaactttgatgtgtgggggcagggcaccacagtgaccgtcagctccggaggaggaggctctggaggaggagggagtggcggaggaggatcagacatccagatgacacagagcccttcaagcctgagcgcctccgtcggtgacagagtgaccattacctgccacgcctcccagaatatctacgtgtggctgaactggtatcagcagaagccaggcaaagcacccaagctgctgatctacaaagccagcaatctgcacaccggagtcccaagcagattctccggttctggcagtggaacagactttaccctgacaatcagcagcctccagcctgaggatttcgcaacttactattgccagcagggccagacatacccatatacttttggcggagggaccaaagtggagatcaagcggtag

SEQ ID NO: 46 - protein, 5 aa, synthetic construct
SYVMH

SEQ ID NO: 47 - protein, 17 aa, synthetic construct
YINPYNDGTKYNEKFQG

SEQ ID NO: 48 - protein, 12 aa, synthetic construct
GTYYYGTRVFDY

SEQ ID NO: 49 - protein, 16 aa, synthetic construct
RSSKSLQNVNGNTYLY

SEQ ID NO: 50 - protein, 7 aa, synthetic construct
RMSNLNS

SEQ ID NO: 51 - protein, 9 aa, synthetic construct
MQHLEYPIT

SEQ ID NO: 52 - protein, 121 aa, synthetic construct
EVQLVESGGGLVKPGGSLKLSCAASGYTFTSYVMHWVRQAPGKGLEWIGYINPYNDGTKYNEKFQGRVTISSDKSISTAYMELSSLRSEDTAMYYCARGTYYYGTRVFDYWGQGTLVTVSS

SEQ ID NO: 53 - DNA, 363 bp, synthetic construct
  source 1..363: mol_type = other DNA
gaggtgcagctggtggagagcggcggcggactggtgaagcctggcggaagcctgaagctgagctgtgccgcctccggctacacctttacctcctacgtgatgcactgggtgaggcaggcccccggcaagggactggagtggatcggctacatcaatccctacaatgatggcacaaagtacaatgagaagtttcagggcagggtgaccatcagctccgataagagcatctccaccgcctacatggagctgtccagcctgagatccgaggataccgccatgtactactgtgccaggggcacctactactacggcacaagggtgttcgactactggggccagggcacactggtgacagtgtcctcc

SEQ ID NO: 54 - protein, 112 aa, synthetic construct
DIVMTQSPATLSLSPGERATLSCRSSKSLQNVNGNTYLYWFQQKPGQSPQLLIYRMSNLNSGVPDRFSGSGSGTEFTLTISSLEPEDFAVYYCMQHLEYPITFGAGTKLEIK

SEQ ID NO: 55 - DNA, 336 bp, synthetic construct
  source 1..336: mol_type = other DNA
gacatcgtgatgacacagagccctgccaccctgagcctgagccccggagagagggccaccctgtcctgtaggtccagcaagagcctgcagaacgtcaatggcaatacatacctgtactggttccagcagaagcctggccagtccccccagctgctgatctacaggatgagcaatctgaacagcggcgtgcctgataggttcagcggctccggcagcggcaccgagttcaccctgaccatcagcagcctggagcccgaggatttcgccgtgtactactgcatgcagcacctggagtaccccatcacattcggcgccggcaccaagctggagatcaag

SEQ ID NO: 56 - protein, 248 aa, synthetic construct
DIVMTQSPATLSLSPGERATLSCRSSKSLQNVNGNTYLYWFQQKPGQSPQLLIYRMSNLNSGVPDRFSGSGSGTEFTLTISSLEPEDFAVYYCMQHLEYPITFGAGTKLEIKGGGGSGGGGSGGGGSEVQLVESGGGLVKPGGSLKLSCAASGYTFTSYVMHWVRQAPGKGLEWIGYINPYNDGTKYNEKFQGRVTISSDKSISTAYMELSSLRSEDTAMYYCARGTYYYGTRVFDYWGQGTLVTVSS

SEQ ID NO: 57 - protein, 5 aa, synthetic construct
KYAMN

SEQ ID NO: 58 - protein, 19 aa, synthetic construct
RIRSKYNNYATYYADSVKD

SEQ ID NO: 59 - protein, 14 aa, synthetic construct
HGNFGNSYISYWAY

SEQ ID NO: 60 - protein, 14 aa, synthetic construct
GSSTGAVTSGNYPN

SEQ ID NO: 61 - protein, 7 aa, synthetic construct
GTKFLAP

SEQ ID NO: 62 - protein, 9 aa, synthetic construct
VLWYSNRWV

SEQ ID NO: 63 - protein, 125 aa, synthetic construct
EVQLVESGGGLVQPGGSLKLSCAASGFTFNKYAMNWVRQAPGKGLEWVARIRSKYNNYATYYADSVKDRFTISRDDSKNTAYLQMNNLKTEDTAVYYCVRHGNFGNSYISYWAYWGQGTLVTVSS

SEQ ID NO: 64 - DNA, 375 bp, synthetic construct
  source 1..375: mol_type = other DNA
gaggtgcaactggttgagagcggcggcggtctggtgcagcccggaggatctctgaagctgagctgtgccgccagcggctttacattcaacaagtacgccatgaattgggtgaggcaggcccccggaaagggcctggagtgggtggctaggatcaggtccaagtacaacaattacgccacatactacgccgattccgtgaaggacaggttcacaatcagcagagacgactccaagaataccgcctacctgcaaatgaataacctgaagaccgaggacacagccgtgtactactgcgtgaggcacggcaattttggcaacagctacatcagctactgggcctactggggccagggaacactggtgaccgtgagcagc

SEQ ID NO: 65 - protein, 109 aa, synthetic construct
QTVVTQEPSLTVSPGGTVTLTCGSSTGAVTSGNYPNWVQQKPGQAPRGLIGGTKFLAPGTPARFSGSLLGGKAALTLSGVQPEDEAEYYCVLWYSNRWVFGGGTKLTVL

SEQ ID NO: 66 - DNA, 327 bp, synthetic construct
  source 1..327: mol_type = other DNA
cagacagtggtgacacaggagccctccctgaccgtgagccccggaggaacagtgaccctgacctgcggcagctccacaggcgccgtgacaagcggcaactaccccaattgggtgcagcagaagcccggccaggccccaaggggactgatcggaggcaccaagttcctggcccctggcacccctgccagattctccggcagcctgctgggcggcaaggccgctctgacactgtccggcgtgcagcccgaggatgaggccgaatactactgcgtcctgtggtacagcaacagatgggtgttcggcggcggcaccaagctcacagtgctg

SEQ ID NO: 67 - protein, 249 aa, synthetic construct
EVQLVESGGGLVQPGGSLKLSCAASGFTFNKYAMNWVRQAPGKGLEWVARIRSKYNNYATYYADSVKDRFTISRDDSKNTAYLQMNNLKTEDTAVYYCVRHGNFGNSYISYWAYWGQGTLVTVSSGGGGSGGGGSGGGGSQTVVTQEPSLTVSPGGTVTLTCGSSTGAVTSGNYPNWVQQKPGQAPRGLIGGTKFLAPGTPARFSGSLLGGKAALTLSGVQPEDEAEYYCVLWYSNRWVFGGGTKLTVL

SEQ ID NO: 68 - protein, 783 aa, synthetic construct
DIVMTQSPATLSLSPGERATLSCRSSKSLQNVNGNTYLYWFQQKPGQSPQLLIYRMSNLNSGVPDRFSGSGSGTEFTLTISSLEPEDFAVYYCMQHLEYPITFGAGTKLEIKGGGGSGGGGSGGGGSEVQLVESGGGLVKPGGSLKLSCAASGYTFTSYVMHWVRQAPGKGLEWIGYINPYNDGTKYNEKFQGRVTISSDKSISTAYMELSSLRSEDTAMYYCARGTYYYGTRVFDYWGQGTLVTVSSGGGGSEVQLVESGGGLVQPGGSLKLSCAASGFTFNKYAMNWVRQAPGKGLEWVARIRSKYNNYATYYADSVKDRFTISRDDSKNTAYLQMNNLKTEDTAVYYCVRHGNFGNSYISYWAYWGQGTLVTVSSGGGGSGGGGSGGGGSQTVVTQEPSLTVSPGGTVTLTCGSSTGAVTSGNYPNWVQQKPGQAPRGLIGGTKFLAPGTPARFSGSLLGGKAALTLSGVQPEDEAEYYCVLWYSNRWVFGGGTKLTVLRNTGRGGEEKKKEKEKEEQEERETKTPESPSHTQPLGVQVQLVQSGAEVKKPGASVKVSCKASGYTFTSYYIHWVRQAPGQGLEWIGCIYPGNVNTNYNEKFKDRATLTVDTSISTAYMELSRLRSDDTAVYFCTRSHYGLDWNFDVWGQGTTVTVSSGGGGSGGGGSGGGGSDIQMTQSPSSLSASVGDRVTITCHASQNIYVWLNWYQQKPGKAPKLLIYKASNLHTGVPSRFSGSGSGTDFTLTISSLQPEDFATYYCQQGQTYPYTFGGGTKVEIKR

SEQ ID NO: 69 - DNA, 2418 bp, synthetic construct
  source 1..2418: mol_type = other DNA
atggacatgagggtccccgctcagctcctggggctcctgctactctggctccgaggtgccagatgtgacatcgtgatgacacagagccctgccaccctgagcctgagccccggagagagggccaccctgtcctgtaggtccagcaagagcctgcagaacgtcaatggcaatacatacctgtactggttccagcagaagcctggccagtccccccagctgctgatctacaggatgagcaatctgaacagcggcgtgcctgataggttcagcggctccggcagcggcaccgagttcaccctgaccatcagcagcctggagcccgaggatttcgccgtgtactactgcatgcagcacctggagtaccccatcacattcggcgccggcaccaagctggagatcaagggcggcggcggcagcggaggaggaggaagcggaggaggcggctccgaggtgcagctggtggagagcggcggcggactggtgaagcctggcggaagcctgaagctgagctgtgccgcctccggctacacctttacctcctacgtgatgcactgggtgaggcaggcccccggcaagggactggagtggatcggctacatcaatccctacaatgatggcacaaagtacaatgagaagtttcagggcagggtgaccatcagctccgataagagcatctccaccgcctacatggagctgtccagcctgagatccgaggataccgccatgtactactgtgccaggggcacctactactacggcacaagggtgttcgactactggggccagggcacactggtgacagtgtcctccggtggcggagggtccgaggtgcaactggttgagagcggcggcggtctggtgcagcccggaggatctctgaagctgagctgtgccgccagcggctttacattcaacaagtacgccatgaattgggtgaggcaggcccccggaaagggcctggagtgggtggctaggatcaggtccaagtacaacaattacgccacatactacgccgattccgtgaaggacaggttcacaatcagcagagacgactccaagaataccgcctacctgcaaatgaataacctgaagaccgaggacacagccgtgtactactgcgtgaggcacggcaattttggcaacagctacatcagctactgggcctactggggccagggaacactggtgaccgtgagcagcggcggcggcggcagcggaggaggaggcagcggaggcggaggaagccagacagtggtgacacaggagccctccctgaccgtgagccccggaggaacagtgaccctgacctgcggcagctccacaggcgccgtgacaagcggcaactaccccaattgggtgcagcagaagcccggccaggccccaaggggactgatcggaggcaccaagttcctggcccctggcacccctgccagattctccggcagcctgctgggcggcaaggccgctctgacactgtccggcgtgcagcccgaggatgaggccgaatactactgcgtcctgtggtacagcaacagatgggtgttcggcggcggcaccaagctcacagtgctgagaaataccggcagaggcggagaggagaagaagaaggagaaggagaaggaggagcaggaggagagagagaccaagacacccgagtctcctagccacacacagcctctgggagtgcaggtgcagctggtccagtcaggagcagaagtcaaaaaacccggcgcatcagtcaaagtctcttgtaaagcctccggatacacatttacatcctactatatccactgggtcagacaggcacctggccagggactggagtggatcggctgcatttacccaggaaacgtgaacaccaactacaacgaaaagttcaaggaccgcgctactctgaccgtcgatacatcaattagcactgcatacatggagctgtctcggctgaggagtgacgatacagctgtgtacttctgtactcgatctcattatggcctggactggaactttgatgtgtgggggcagggcaccacagtgaccgtcagctccggaggaggaggctctggaggaggagggagtggcggaggaggatcagacatccagatgacacagagcccttcaagcctgagcgcctccgtcggtgacagagtgaccattacctgccacgcctcccagaatatctacgtgtggctgaactggtatcagcagaagccaggcaaagcacccaagctgctgatctacaaagccagcaatctgcacaccggagtcccaagcagattctccggttctggcagtggaacagactttaccctgacaatcagcagcctccagcctgaggatttcgcaacttactattgccagcagggccagacatacccatatacttttggcggagggaccaaagtggagatcaagcggtag